European Patent Specification EP 3 242 895 B1, published March 12, 2025. Title: A NOVEL ANTI-EGFR MONOCLONAL ANTIBODY, METHOD OF MAKING, AND USE THEREOF. Applicant: SHANGHAI ZHANGJIANG BIOTECHNOLOGY CO., LTD. The sequence listing filed with the application follows.

SEQUENCE LISTING (14 sequences)

SEQ ID NO: 1 - DNA, 642 bp, Artificial sequence
  misc_feature: cetuximab light chain
gatatccttctgacacagtctccagtgatactgtcagtttctccaggggagcgcgtctcatttagttgtcgggccagtcagagtatcggcacaaacatccattggtaccagcagcggacaaacggctccccccggttgctcattaagtacgcaagcgagtctatctctgggataccaagtcgcttctcgggtagtggtagcggaacagattttactctgagtatcaatagcgtcgaatccgaagatattgccgattactactgtcagcagaataacaactggccaaccacattcggcgccggtaccaagctggaactcaagcgcacagttgccgcacctagtgtcttcatcttcccaccatctgacgagcaactaaagagtggcactgcaagtgtcgtatgtctgctgaacaacttttacccacgggaggctaaagtgcagtggaaggtagacaacgcccttcagagcggaaattctcaggaaagcgtcaccgaacaagattccaaggatagcacatactccctgtcctctaccctgacactgtcaaaagctgactacgaaaagcataaagtgtatgcttgcgaggtgactcatcaggggctcagctcgcccgtcaccaagtccttcaaccgtggagaatgt

SEQ ID NO: 2 - protein, 214 aa, Artificial sequence
  MISC_FEATURE: cetuximab light chain
DILLTQSPVILSVSPGERVSFSCRASQSIGTNIHWYQQRTNGSPRLLIKYASESISGIPSRFSGSGSGTDFTLSINSVESEDIADYYCQQNNNWPTTFGAGTKLELKRTVAAPSVFIFPPSDEQLKSGTASVVCLLNNFYPREAKVQWKVDNALQSGNSQESVTEQDSKDSTYSLSSTLTLSKADYEKHKVYACEVTHQGLSSPVTKSFNRGEC

SEQ ID NO: 3 - DNA, 1347 bp, Artificial sequence
  misc_feature: cetuximab heavy chain
caggtgcagctgaagcagagcggaccaggcctggtccagccctcacagtccctgagcattacttgtactgtgagtgggttctcgttgacgaactacggggtgcattgggtgcgccagagtcccggtaaagggctggagtggttaggcgtgatttggagcggcggtaacactgactataatacccctttcaccagtcgcttgagtatcaataaggataattcaaagtctcaagtgttttttaagatgaactccctacagagcaacgatacggctatctactactgtgcccgcgcccttacatactacgactatgagttcgcttattggggccaggggaccttggtcactgtgtctgcagcttctacaaaagggccatccgtgttcccactggcccccagttccaagagcactagtggtggcacagcagccctcgggtgcctcgtgaaggattacttcccggagccagtgaccgtcagttggaactccggcgctctaacaagcggagtacatacttttccagccgtgctgcagtcttcagggctttacagtctttcctccgttgtgacagtgcccagcagcagcctgggcacccagacttatatttgtaatgtgaaccataagccttctaatactaaggtggacaagagagttgagccaaagtcctgtgacaaaactcacacatgccccccttgcccagctcctgagttgttgggcggcccttccgtcttcctgtttcccccgaaacctaaggataccctgatgatatctcggacaccagaagtgacatgcgtcgtggtcgatgtgtcacacgaagaccctgaggtgaaatttaactggtacgtagacggtgtagaagttcacaacgctaagacaaagcctcgggaagagcagtacaactcaacctaccgagtagtgtccgtgcttactgttctgcaccaggactggctgaatggaaaggaatataagtgtaaagtgtccaataaggcactgcctgctccaatcgagaagacgatttctaaagccaagggacaaccaagagaacctcaggtgtataccttgcccccatctagagaagagatgaccaaaaaccaggtgtcacttacatgcctcgtgaaaggcttctatccttctgacattgccgtcgaatgggagagtaacggacagcccgagaacaactacaagaccacacctccagtgctggattcggatggctctttcttcctttatagtaagctcactgtggacaagtcccgatggcagcaggggaacgtgttctcttgcagcgtgatgcacgaggcattgcataatcactacacccagaagtctctctcattatcccctggcaag

SEQ ID NO: 4 - protein, 449 aa, Artificial sequence
  MISC_FEATURE: cetuximab heavy chain
QVQLKQSGPGLVQPSQSLSITCTVSGFSLTNYGVHWVRQSPGKGLEWLGVIWSGGNTDYNTPFTSRLSINKDNSKSQVFFKMNSLQSNDTAIYYCARALTYYDYEFAYWGQGTLVTVSAASTKGPSVFPLAPSSKSTSGGTAALGCLVKDYFPEPVTVSWNSGALTSGVHTFPAVLQSSGLYSLSSVVTVPSSSLGTQTYICNVNHKPSNTKVDKRVEPKSCDKTHTCPPCPAPELLGGPSVFLFPPKPKDTLMISRTPEVTCVVVDVSHEDPEVKFNWYVDGVEVHNAKTKPREEQYNSTYRVVSVLTVLHQDWLNGKEYKCKVSNKALPAPIEKTISKAKGQPREPQVYTLPPSREEMTKNQVSLTCLVKGFYPSDIAVEWESNGQPENNYKTTPPVLDSDGSFFLYSKLTVDKSRWQQGNVFSCSVMHEALHNHYTQKSLSLSPGK

SEQ ID NO: 5 - protein, 108 aa, Artificial sequence
  MISC_FEATURE: variable region of light chain
DILLTQSPVILSVSPGERVSFSCRASQSIGTNIHWYQQRTNGSPRLLIKYASESISGIPSRFSGSGSGTDFTLSINSVESEDIADYYCQQNNNWPTTFGAGTKLELKR

SEQ ID NO: 6 - protein, 11 aa, Artificial sequence
  MISC_FEATURE: CDR1 of light chain
RASQSIGTNIH

SEQ ID NO: 7 - protein, 7 aa, Artificial sequence
  MISC_FEATURE: CDR2 of light chain
YASESIS

SEQ ID NO: 8 - protein, 9 aa, Artificial sequence
  MISC_FEATURE: CDR3 of light chain
QQNNNWPTT

SEQ ID NO: 9 - protein, 119 aa, Artificial sequence
  variable region of light chain
QVQLKQSGPGLVQPSQSLSITCTVSGFSLTNYGVHWVRQSPGKGLEWLGVIWSGGNTDYNTPFTSRLSINKDNSKSQVFFKMNSLQSNDTAIYYCARALTYYDYEFAYWGQGTLVTVSA

SEQ ID NO: 10 - protein, 5 aa, Artificial sequence
  MISC_FEATURE: CDR1 of heavy chain
NYGVH

SEQ ID NO: 11 - protein, 16 aa, Artificial sequence
  MISC_FEATURE: CDR2 of heavy chain
VIWSGGNTDYNTPFTS

SEQ ID NO: 12 - protein, 11 aa, Artificial sequence
  MISC_FEATURE: CDR3 of heavy chain
ALTYYDYEFAY

SEQ ID NO: 13 - protein, 25 aa, Artificial sequence
  MISC_FEATURE: Signal peptide
MATMVPSSVPCHWLLFLLLLFSGSS

SEQ ID NO: 14 - DNA, 75 bp, Artificial sequence
  misc_feature: Signal peptide
atggccaccatggtgccctcttctgtgccctgccactggctgctgttcctgctgctgctgttctctggctcttct